European Patent Application EP 4 527 930 A1, published March 26, 2025. Title: COMPOSITION FOR TREATMENT OF SEPSIS BY REGULATING OLFR164. Applicant: Daegu Gyeongbuk Institute of Science and Technology. The sequence listing filed with the application follows.

SEQUENCE LISTING (5 sequences)

SEQ ID NO: 1 - DNA, 20 bp, synthetic construct
  source 1..20: mol_type = other DNA
ccatgtacatccttctcagc

SEQ ID NO: 2 - DNA, 22 bp, synthetic construct
  source 1..22: mol_type = other DNA
gaagaatatctggattccacag

SEQ ID NO: 3 - DNA, 942 bp, synthetic construct
  source 1..942: mol_type = other DNA
atgatacaatggaacaactggaccaggaactctgatttcatcctactaggattatttgatcacagtcctcttcatacttttttcttttccctaattctgggtatcttcttcatggccttcataggaaattctatcatggtgattctcatctacttggatgctcatctccacacccccatgtacatccttctcagccaactttctctcatggatctcatgctcatctgtactacagtaccccaaatggccttcaacttcctttctggaaacaagtccatctccatggttggctgtggaatccagatattcttctatgtatctctacttggagctgagtgttttttgttggccgcaatggcttatgaccgttatgtagctatttgctacccattaaggtaccctattctcatgagtgacaaaatatgtggcctcatggctgcctcctcttgggttcttggctctcttgatggtataatagaagttgcagctgcattgtctttttcatattgtggtgccagagaaatacctcattttttctgtgatgttcctgccttactcacactttcatgtagtaataccttgatatttgaaagaattatatttttctgctgtgtaattatgcttactttacctgtagcaatcattattgcttcctatactcgtgtgattctgaccgttcttcatatgagctcagctgagagtcgccacaaagcttttgccacctgttcctctcacctcatggtggtgggaatgtactatggggcagccatgttcatatacatgcggccttcttctggtcgttctcccacccaggacaaaatagtgtcagctttctacactatccttacgccaatgttgaaccccctcatttatagtctccggaacaaagaagtagccagagcattcatgaaagtgttagggattgataaggcagcagcatga

SEQ ID NO: 4 - DNA, 931 bp, synthetic construct
  source 1..931: mol_type = other DNA
atgatacaatggaacaactggaccaggaactctgatttcatcctactaggattatttgatcacagtcctcttcatacttttttcttttccctaattctgggtatcttcttcatggccttcataggaaattctatcatggtgattctcatctacttggatgctcatctccacacccccatgtacatccttctcagccaactttctctcatggatctcatgctcatctgtactacagtaccccaaattcctttctggaaacaagtccatctccatggttggctgtggaatccagatattcttctatgtatctctacttggagctgagtgttttttgttggccgcaatggcttatgaccgttatgtagctatttgctacccattaaggtaccctattctcatgagtgacaaaatatgtggcctcatggctgcctcctcttgggttcttggctctcttgatggtataatagaagttgcagctgcattgtctttttcatattgtggtgccagagaaatacctcattttttctgtgatgttcctgccttactcacactttcatgtagtaataccttgatatttgaaagaattatatttttctgctgtgtaattatgcttactttacctgtagcaatcattattgcttcctatactcgtgtgattctgaccgttcttcatatgagctcagctgagagtcgccacaaagcttttgccacctgttcctctcacctcatggtggtgggaatgtactatggggcagccatgttcatatacatgcggccttcttctggtcgttctcccacccaggacaaaatagtgtcagctttctacactatccttacgccaatgttgaaccccctcatttatagtctccggaacaaagaagtagccagagcattcatgaaagtgttagggattgataaggcagcagcatga

SEQ ID NO: 5 - DNA, 22 bp, synthetic construct
  source 1..22: mol_type = other DNA
ccccaaatggccttcaacttcc